European Patent Application EP 4 700 043 A1, published February 25, 2026. Title: Insecticidal peptide from venom of scorpion. Applicant: 国立大学法人京都大学. The sequence listing filed with the application follows.

SEQUENCE LISTING (21 sequences)

SEQ ID NO: 1 - protein, 24 aa, Liocheles australasiae
  DISULFID 4..22: note = Intrachain difulfide bridge
  DISULFID 8..18: note = Intrachain disulfide bridge
GNSCMEVCLQHEGNVAECEKACNK

SEQ ID NO: 2 - protein, 25 aa, Liocheles australasiae
  DISULFID 4..22: note = Intrachain difulfide bridge
  DISULFID 8..18: note = Intrachain disulfide bridge
DSACVEVCLHHEGNVAECEEACKKS

SEQ ID NO: 3 - protein, 23 aa, Liocheles australasiae
  DISULFID 6..21: note = Intrachain disulfide bridge
  DISULFID 10..17: note = Intrachain disulfide bridge
LVQKPCRIVCSENMRKCIRRCTL

SEQ ID NO: 4 - protein, 24 aa, Liocheles australasiae
  DISULFID 6..24: note = Intrachain disulfide bridge
  DISULFID 10..20: note = Intrachain disulfide bridge
AERAGCRIRCLQFTDDFEKCRKLC

SEQ ID NO: 5 - protein, 23 aa, Liocheles australasiae
  DISULFID 2..19: note = Intrachain disulfide bridge
  DISULFID 6..15: note = Intrachain disulfide bridge
SCKRVCSGTRRTKKCMQKCKSQP

SEQ ID NO: 6 - protein, 26 aa, Opisthacanthus madagascariensis
  DISULFID 3..21: note = Intrachain disulfide bridge
  DISULFID 7..17: note = Intrachain disulfide bridge
DPCYEVCLQQHGNVKECEEACKHPVE

SEQ ID NO: 7 - protein, 24 aa, Synthetic construct
  DISULFID 4..22: note = Intrachain disulfide bridge
  DISULFID 8..18: note = Intrachain disulfide bridge
GNSCMEVCLHHEGNVAECEKACNK

SEQ ID NO: 8 - protein, 25 aa, Synthetic construct
  DISULFID 4..22: note = Intrachain disulfide bridge
  DISULFID 8..18: note = Intrachain disulfide bridge
DSACVEVCLQHEGNVAECEEACKKS

SEQ ID NO: 9 - protein, 25 aa, Synthetic construct
  DISULFID 4..22: note = Intrachain disulfide bridge
  DISULFID 8..18: note = Intrachain disulfide bridge
DSACVAVCLHHEGNVAECEEACKKS

SEQ ID NO: 10 - protein, 25 aa, Synthetic construct
  DISULFID 4..22: note = Intrachain disulfide bridge
  DISULFID 8..18: note = Intrachain disulfide bridge
DSACVEVCLHHAGNVAECEEACKKS

SEQ ID NO: 11 - protein, 25 aa, Synthetic construct
  DISULFID 4..22: note = Intrachain disulfide bridge
  DISULFID 8..18: note = Intrachain disulfide bridge
DSACVEVCLHHEGNVAECEKACKKS

SEQ ID NO: 12 - DNA, 75 bp, Liocheles australasiae
  source 1..75: mol_type = genomic DNA
gattcggcttgtgtggaagtgtgccttcatcatgaaggaaatgtagcagagtgtgaagaagcatgcaaaaagagc

SEQ ID NO: 13 - DNA, 69 bp, Liocheles australasiae
  source 1..69: mol_type = genomic DNA
tcgtgcaaaagagtgtgctcggggaccagacgcacgaaaaaatgcatgcagaagtgtaaatcacagcct

SEQ ID NO: 14 - DNA, 72 bp, Synthetic construct
  source 1..72: mol_type = other DNA
ggtaattcctgtatggaagtgtgccttcatcatgaaggaaatgtagcagagtgtgaaaaagcatgcaataag

SEQ ID NO: 15 - protein, 25 aa, Synthetic construct
ASACVEVCLHHEGNVAECEEACKKS

SEQ ID NO: 16 - protein, 25 aa, Synthetic construct
DSACVEVCLHAEGNVAECEEACKKS

SEQ ID NO: 17 - protein, 25 aa, Synthetic construct
DSACVEVCLHHEGNVAACEEACKKS

SEQ ID NO: 18 - protein, 25 aa, Synthetic construct
DSACVEVCLHHEGNVAECAEACKKS

SEQ ID NO: 19 - protein, 25 aa, Synthetic construct
DSACVEVCLHHEGNVAECEAACKKS

SEQ ID NO: 20 - protein, 25 aa, Synthetic construct
DSACVEVCLHHEGNVAECEEACAKS

SEQ ID NO: 21 - protein, 25 aa, Synthetic construct
DSACVEVCLHHEGNVAECEEACKAS